European Patent Specification EP 4 090 768 B1, published March 13, 2024. Title: COMPOSITIONS, KITS AND METHODS FOR ISOLATING TARGET POLYNUCLEOTIDES. Applicant: DNAe DIAGNOSTICS LIMITED NELSON, Norm WOOLDRIDGE, David. The sequence listing filed with the application follows.

SEQUENCE LISTING (36 sequences)

SEQ ID NO: 1 - DNA, 24 bp, Artificial Sequence
  Synthetic
gtatcagcgcgaagtctttatacc

SEQ ID NO: 2 - DNA, 24 bp, Artificial Sequence
  Synthetic
ggcaataacatacggagtgacatc

SEQ ID NO: 3 - DNA, 169 bp, Artificial Sequence
  Synthetic
gtatcagcgcgaagtctttataccgaaaggttgggcgggccagcgtattgtactgcgtttcgatgcggtcactcattacggcaaagtgtgggtaaataatcaggaagtgatggagcatcagggcggctatacgccatttgaagccgatgtcactccgtatgttattgcc

SEQ ID NO: 4 - DNA, 128 bp, Artificial Sequence
  Synthetic
  misc_feature (41)..(42): site of iSp18 (Hexaethylene Glycol (HEG) internal spacer )
aaaaaaaaaaaaaaaaaaaaaaaaaaaaaaaaaaacctctatttttttttttttttttttttttttttttttttttagacgcaagctactggtgatttggcaataacatacggagtgacatcggcttc

SEQ ID NO: 5 - DNA, 22 bp, Artificial Sequence
  Synthetic
agacgcaagctactggtgattt

SEQ ID NO: 6 - DNA, 30 bp, Artificial Sequence
  Synthetic
ggcaataacatacggagtgacatcggcttc

SEQ ID NO: 7 - DNA, 20 bp, Artificial Sequence
  Synthetic
  misc_feature: 3' Biotin
tttttttttttttttttttt

SEQ ID NO: 8 - DNA, 29 bp, Artificial Sequence
  Synthetic
  misc_feature: 5' FAM, 3' IowaBlack
tagccgccctgatgctccatcacttcctg

SEQ ID NO: 9 - DNA, 20 bp, Artificial Sequence
  Synthetic
agacgcaagctactggtgat

SEQ ID NO: 10 - DNA, 22 bp, Artificial Sequence
  Synthetic
ggctgcgatattcaaagctcag

SEQ ID NO: 11 - DNA, 19 bp, Artificial Sequence
  Synthetic
ctgaacgcgccggcttaac

SEQ ID NO: 12 - DNA, 166 bp, Artificial Sequence
  Synthetic
ggctgcgatattcaaagctcagcaatttgtatggacaaatcgttgacatacatcgttgcgaaaaatgctgggatagctactcccgccttttgggttattaataaagatgataggccggtggcagctacgtttacctatcctgtttttgttaagccggcgcgttcag

SEQ ID NO: 13 - DNA, 77 bp, Artificial Sequence
  Synthetic
  misc_feature (20)..(21): site of iSp18 (Hexaethylene Glycol (HEG) internal spacer )
aaaaaaaaaaaaaaaaaaaactcctctggcaccgtgctgccttggcttcattgtggtcctgaacgcgccggcttaac

SEQ ID NO: 14 - DNA, 38 bp, Artificial Sequence
  Synthetic
ctcctctggcaccgtgctgccttggcttcattgtggtc

SEQ ID NO: 15 - DNA, 19 bp, Artificial Sequence
  Synthetic
ctgaacgcgccggcttaac

SEQ ID NO: 16 - DNA, 24 bp, Artificial Sequence
  Synthetic
  misc_feature: 3' invdt
cggtgccagaggagtttttttttt

SEQ ID NO: 17 - DNA, 14 bp, Artificial Sequence
  Synthetic
cggtgccagaggag

SEQ ID NO: 18 - DNA, 10 bp, Artificial Sequence
  Synthetic
tttttttttt

SEQ ID NO: 19 - DNA, 20 bp, Artificial Sequence
  Synthetic
  misc_feature: 3' Biotin
tttttttttttttttttttt

SEQ ID NO: 20 - DNA, 26 bp, Artificial Sequence
  Synthetic
ttgtatggacaaatcgttgacataca

SEQ ID NO: 21 - DNA, 28 bp, Artificial Sequence
  Synthetic
  misc_feature: 5' FAM, 3' IowaBlack
tgctgggatagctactcccgccttttgg

SEQ ID NO: 22 - DNA, 19 bp, Artificial Sequence
  Synthetic
accgtgctgccttggcttc

SEQ ID NO: 23 - DNA, 22 bp, Artificial Sequence
  Synthetic
ggctgcgatattcaaagctcag

SEQ ID NO: 24 - DNA, 19 bp, Artificial Sequence
  Synthetic
ctgaacgcgccggcttaac

SEQ ID NO: 25 - DNA, 166 bp, Artificial Sequence; identical to SEQ ID NO: 12
  Synthetic

SEQ ID NO: 26 - DNA, 77 bp, Artificial Sequence
  Synthetic
  misc_feature (20)..(21): site of iSp18 (Hexaethylene Glycol (HEG) internal spacer )
aaaaaaaaaaaaaaaaaaaactcctctggcaccgtgctgccttggcttcattgtggtcgtagctgccaccggcctat

SEQ ID NO: 27 - DNA, 38 bp, Artificial Sequence; identical to SEQ ID NO: 14
  Synthetic

SEQ ID NO: 28 - DNA, 19 bp, Artificial Sequence
  Synthetic
gtagctgccaccggcctat

SEQ ID NO: 29 - DNA, 24 bp, Artificial Sequence
  Synthetic
  misc_feature: 3' invdt
cggtgccagaggagtttttttttt

SEQ ID NO: 30 - DNA, 14 bp, Artificial Sequence
  Synthetic
cggtgccagaggag

SEQ ID NO: 31 - DNA, 10 bp, Artificial Sequence
  Synthetic
tttttttttt

SEQ ID NO: 32 - DNA, 47 bp, Artificial Sequence
  Synthetic
aaaacgagacatgccgagcatccgcggctgcgatattcaaagctcag

SEQ ID NO: 33 - DNA, 20 bp, Artificial Sequence
  Synthetic
  misc_feature: 3' Biotin
tttttttttttttttttttt

SEQ ID NO: 34 - DNA, 22 bp, Artificial Sequence
  Synthetic
aaaacgagacatgccgagcatc

SEQ ID NO: 35 - DNA, 28 bp, Artificial Sequence
  Synthetic
  misc_feature: 5' FAM, 3' IowaBlack
tgctgggatagctactcccgccttttgg

SEQ ID NO: 36 - DNA, 19 bp, Artificial Sequence
  Synthetic
accgtgctgccttggcttc